European Patent Specification EP 3 209 772 B1, published December 11, 2024. Title: Mutated Fucosidase. Applicant: Glycom A/S. The sequence listing filed with the application follows.

SEQUENCE LISTING (1 sequence)

SEQ ID NO: 1 - protein, 478 aa, Bifidobacterium longum subsp. infantis
MNNPADAGINLNYLANVRPSSRQLAWQRMEMYAFLHFGMNTMTDREWGLGHEDPALFNPRNVDVDQWMDALVAGGMAGVILTCKHHDGFCLWPSRLTRHTVASSPWREGKGDLVREVSESARRHGLKFGVYLSPWDRTEESYGKGKAYDDFYVGQLTELLTQYGPIFSVWLDGANGEGKNGKTQYYDWDRYYNVIRSLQPDAVISVCGPDVRWAGNEAGHVRDNEWSVVPRRLRSAELTMEKSQQEDDASFATTVSSQDDDLGSREAVAGYGDNVCWYPAEVDTSIRPGWFYHQSEDDKVMSADQLFDLWLSAVGGNSSLLLNIPPSPEGLLAEPDVQSLKGLGRRVSEFREALASVRCEARTSSASAAAAHLVDGNRDTFWRPDADDAAPAITLTLPQPTTINAIVIEEAIEHGQRIEHLRVTGALPDGTERVLGQAGTVGYRRILRFDDVEVSSVTLHVDGSRLAPMISRAAAVRI